European Patent Application EP 4 644 564 A1, published November 5, 2025. Title: DETECTION COMPOSITION AND PROTEIN CAPTURE DETECTION METHOD. Applicant: BGI SHENZHEN. Application EP 22969617.4, filed December 28, 2022. The sequence listing filed with the application follows.

SEQUENCE LISTING (42 sequences)

SEQ ID NO: 1 - DNA, 21 bp, synthetic construct
  source 1..21: mol_type = other DNA
ccttggcacccgagaattcca

SEQ ID NO: 2 - DNA, 31 bp, synthetic construct
  source 1..31: mol_type = other DNA
  modified_base 30..31: mod_base = OTHER; note; note (original language) = thio-modified a
baaaaaaaaaaaaaaaaaaaaaaaaaaaann

SEQ ID NO: 3 - DNA, 15 bp, synthetic construct
  source 1..15: mol_type = other DNA
aacaagacccttgag

SEQ ID NO: 4 - DNA, 15 bp, synthetic construct
  source 1..15: mol_type = other DNA
tacccgtaatagcgt

SEQ ID NO: 5 - DNA, 15 bp, synthetic construct
  source 1..15: mol_type = other DNA
ccctttcacctcgaa

SEQ ID NO: 6 - DNA, 15 bp, synthetic construct
  source 1..15: mol_type = other DNA
aagtcgtgaggcatg

SEQ ID NO: 7 - DNA, 15 bp, synthetic construct
  source 1..15: mol_type = other DNA
tgaaggctcatttgt

SEQ ID NO: 8 - DNA, 15 bp, synthetic construct
  source 1..15: mol_type = other DNA
acattgacgcaacta

SEQ ID NO: 9 - DNA, 15 bp, synthetic construct
  source 1..15: mol_type = other DNA
tggcttcaggtccta

SEQ ID NO: 10 - DNA, 15 bp, synthetic construct
  source 1..15: mol_type = other DNA
gcgcgtttgtgctat

SEQ ID NO: 11 - DNA, 15 bp, synthetic construct
  source 1..15: mol_type = other DNA
ccgatcagccgttta

SEQ ID NO: 12 - DNA, 15 bp, synthetic construct
  source 1..15: mol_type = other DNA
cctacacctcataat

SEQ ID NO: 13 - DNA, 15 bp, synthetic construct
  source 1..15: mol_type = other DNA
ggataatttcgatcc

SEQ ID NO: 14 - DNA, 15 bp, synthetic construct
  source 1..15: mol_type = other DNA
ttaacttcagcccgt

SEQ ID NO: 15 - DNA, 15 bp, synthetic construct
  source 1..15: mol_type = other DNA
ccgcacctacattag

SEQ ID NO: 16 - DNA, 15 bp, synthetic construct
  source 1..15: mol_type = other DNA
gtatgtccgctcgat

SEQ ID NO: 17 - DNA, 15 bp, synthetic construct
  source 1..15: mol_type = other DNA
tccactccctgtata

SEQ ID NO: 18 - DNA, 15 bp, synthetic construct
  source 1..15: mol_type = other DNA
cgttcctacctacct

SEQ ID NO: 19 - DNA, 15 bp, synthetic construct
  source 1..15: mol_type = other DNA
ttcgatgctggagca

SEQ ID NO: 20 - DNA, 15 bp, synthetic construct
  source 1..15: mol_type = other DNA
agctagacacgttgt

SEQ ID NO: 21 - DNA, 15 bp, synthetic construct
  source 1..15: mol_type = other DNA
gagcaagattaagac

SEQ ID NO: 22 - DNA, 15 bp, synthetic construct
  source 1..15: mol_type = other DNA
attgacgacagtcat

SEQ ID NO: 23 - DNA, 15 bp, synthetic construct
  source 1..15: mol_type = other DNA
accgaccagtagaca

SEQ ID NO: 24 - DNA, 15 bp, synthetic construct
  source 1..15: mol_type = other DNA
agctacgcattcaat

SEQ ID NO: 25 - DNA, 15 bp, synthetic construct
  source 1..15: mol_type = other DNA
cgtatccgtctccta

SEQ ID NO: 26 - DNA, 15 bp, synthetic construct
  source 1..15: mol_type = other DNA
gtcattgcggtccta

SEQ ID NO: 27 - DNA, 15 bp, synthetic construct
  source 1..15: mol_type = other DNA
ctttctttcacggga

SEQ ID NO: 28 - DNA, 15 bp, synthetic construct
  source 1..15: mol_type = other DNA
tcatatccgttgtcc

SEQ ID NO: 29 - DNA, 15 bp, synthetic construct
  source 1..15: mol_type = other DNA
gcgagaaatctgcat

SEQ ID NO: 30 - DNA, 15 bp, synthetic construct
  source 1..15: mol_type = other DNA
gcagtcctacattga

SEQ ID NO: 31 - DNA, 15 bp, synthetic construct
  source 1..15: mol_type = other DNA
acgcagtatttccga

SEQ ID NO: 32 - DNA, 15 bp, synthetic construct
  source 1..15: mol_type = other DNA
atttgtatgctggag

SEQ ID NO: 33 - DNA, 15 bp, synthetic construct
  source 1..15: mol_type = other DNA
gctgtagtatcatgt

SEQ ID NO: 34 - DNA, 15 bp, synthetic construct
  source 1..15: mol_type = other DNA
cagctcagtgtgttg

SEQ ID NO: 35 - DNA, 15 bp, synthetic construct
  source 1..15: mol_type = other DNA
atcagccatgtcagt

SEQ ID NO: 36 - DNA, 15 bp, synthetic construct
  source 1..15: mol_type = other DNA
aaccaacagtcacgt

SEQ ID NO: 37 - DNA, 15 bp, synthetic construct
  source 1..15: mol_type = other DNA
aagtcaggttcgttt

SEQ ID NO: 38 - DNA, 108 bp, synthetic construct
  source 1..108: mol_type = other DNA
  modified_base 37..61: mod_base = OTHER; note; note (original language) = n=a,t,c or g
  modified_base 77..86: mod_base = OTHER; note; note (original language) = n=a,t,c or g
ctgctgacgtactgagaggcatggcgaccttatcagnnnnnnnnnnnnnnnnnnnnnnnnnttgtcttcctaagacnnnnnnnnnntttttttttttttttttttttv

SEQ ID NO: 39 - DNA, 36 bp, synthetic construct
  source 1..36: mol_type = other DNA
ctgctgacgtactgagaggcatggcgaccttatcag

SEQ ID NO: 40 - DNA, 22 bp, synthetic construct
  source 1..22: mol_type = other DNA
tttttttttttttttttttttv

SEQ ID NO: 41 - DNA, 22 bp, synthetic construct
  source 1..22: mol_type = other DNA
  modified_base 1: mod_base = OTHER; note; note (original language) = n is phosphorylated c
  modified_base 17: mod_base = OTHER; note; note (original language) = n is thio-modified a
  modified_base 18..19: mod_base = OTHER; note; note (original language) = n is thio-modified g
  modified_base 20: mod_base = OTHER; note; note (original language) = n is thio-modified c
  modified_base 21: mod_base = OTHER; note; note (original language) = n is thio-modified a
  modified_base 22: mod_base = OTHER; note; note (original language) = n is thio-modified t
ctgctgacgtactgagnnnnnn

SEQ ID NO: 42 - DNA, 43 bp, synthetic construct
  source 1..43: mol_type = other DNA
gagacgttctcgactcagcagaccttggcacccgagaattcca